European Patent Specification EP 3 612 623 B1, published July 3, 2024. Title: COMPOSITIONS AND METHODS FOR INCREASING THE CULTURE DENSITY OF A CELLULAR BIOMASS WITHIN A CULTIVATION INFRASTRUCTURE. Applicant: Memphis Meats, Inc. Application PCT/US2018/031276. The sequence listing filed with the application follows.

SEQUENCE LISTING (31 sequences)

SEQ ID NO: 1 - DNA, 1464 bp, Homo sapiens
atggatcccgggcagcagccgccgcctcaaccggccccccagggccaagggcagccgccttcgcagcccccgcaggggcagggcccgccgtccggacccgggcaaccggcacccgcggcgacccaggcggcgccgcaggcaccccccgccgggcatcagatcgtgcacgtccgcggggactcggagaccgacctggaggcgctctttaacgccgtcatgaaccccaagacggccaacgtgccccagaccgtgcccatgaggctccggaagctgcccgactccttcttcaagccgccggagcccaaatcccactcccgacaggccagtactgatgcaggcactgcaggagccctgactccacagcatgttcgagctcatgcctctccagcttctctgcagttgggagctgtttctcctgggacactgacccccactggagtagtctctggcccagcagctacacccacagctcagcatcttcgacagtcttcttttgagatacctgatgatgtacctctgccagcaggttgggagatggcaaagacatcttctggtcagagatacttcttaaatcacatcgatcagacaacaacatggcaggaccccaggaaggccatgctgtcccagatgaacgtcacagcccccaccagtccaccagtgcagcagaatatgatgaactcggcttcaggtcctcttcctgatggatgggaacaagccatgactcaggatggagaaatttactatataaaccataagaacaagaccacctcttggctagacccaaggcttgaccctcgttttgccatgaaccagagaatcagtcagagtgctccagtgaaacagccaccacccctggctccccagagcccacagggaggcgtcatgggtggcagcaactccaaccagcagcaacagatgcgactgcagcaactgcagatggagaaggagaggctgcggctgaaacagcaagaactgcttcggcaggagttagccctgcgtagccagttaccaacactggagcaggatggtgggactcaaaatccagtgtcttctcccgggatgtctcaggaattgagaacaatgacgaccaatagctcagatcctttccttaacagtggcacctatcactctcgagatgagagtacagacagtggactaagcatgagcagctacagtgtccctcgaaccccagatgacttcctgaacagtgtggatgagatggatacaggtgatactatcaaccaaagcaccctgccctcacagcagaaccgtttcccagactaccttgaagccattcctgggacaaatgtggaccttggaacactggaaggagatggaatgaacatagaaggagaggagctgatgccaagtctgcaggaagctttgagttctgacatccttaatgacatggagtctgttttggctgccaccaagctagataaagaaagctttcttacatggtta

SEQ ID NO: 2 - DNA, 1467 bp, Homo sapiens
  ref <308>: NCBI/NM_001195044.1
  ref <309>: 2018-03-29
  ref <313>: (1)..(1467)
atggatcccgggcagcagccgccgcctcaaccggccccccagggccaagggcagccgccttcgcagcccccgcaggggcagggcccgccgtccggacccgggcaaccggcacccgcggcgacccaggcggcgccgcaggcaccccccgccgggcatcagatcgtgcacgtccgcggggactcggagaccgacctggaggcgctcttcaacgccgtcatgaaccccaagacggccaacgtgccccagaccgtgcccatgaggctccggaagctgcccgactccttcttcaagccgccggagcccaaatcccactcccgacaggccagtactgatgcaggcactgcaggagccctgactccacagcatgttcgagctcattcctctccagcttctctgcagttgggagctgtttctcctgggacactgacccccactggagtagtctctggcccagcagctacacccacagctcagcatcttcgacagtcttcttttgagatacctgatgatgtacctctgccagcaggttgggagatggcaaagacatcttctggtcagagatacttcttaaatcacatcgatcagacaacaacatggcaggaccccaggaaggccatgctgtcccagatgaacgtcacagcccccaccagtccaccagtgcagcagaatatgatgaactcggcttcaggtcctcttcctgatggatgggaacaagccatgactcaggatggagaaatttactatataaaccataagaacaagaccacctcttggctagacccaaggcttgaccctcgttttgccatgaaccagagaatcagtcagagtgctccagtgaaacagccaccacccctggctccccagagcccacagggaggcgtcatgggtggcagcaactccaaccagcagcaacagatgcgactgcagcaactgcagatggagaaggagaggctgcggctgaaacagcaagaactgcttcggcaggagttagccctgcgtagccagttaccaacactggagcaggatggtgggactcaaaatccagtgtcttctcccgggatgtctcaggaattgagaacaatgacgaccaatagctcagatcctttccttaacagtggcacctatcactctcgagatgagagtacagacagtggactaagcatgagcagctacagtgtccctcgaaccccagatgacttcctgaacagtgtggatgagatggatacaggtgatactatcaaccaaagcaccctgccctcacagcagaaccgtttcccagactaccttgaagccattcctgggacaaatgtggaccttggaacactggaaggagatggaatgaacatagaaggagaggagctgatgccaagtctgcaggaagctttgagttctgacatccttaatgacatggagtctgttttggctgccaccaagctagataaagaaagctttcttacatggttatag

SEQ ID NO: 3 - DNA, 1200 bp, Homo sapiens
atgaatccggcctcggcgccccctccgctcccgccgcctgggcagcaagtgatccacgtcacgcaggacctagacacagacctcgaagccctcttcaactctgtcatgaatccgaagcctagctcgtggcggaagaagatcctgccggagtctttctttaaggagcctgattcgggctcgcactcgcgccagtccagcaccgactcgtcgggcggccacccggggcctcgactggctgggggtgcccagcatgtccgctcgcacgcgtcgcccgcgtccctgcagctgggcaccggcgcgggtgctgcgggtagccccgcgcagcagcacgcgcacctccgccagcagtcctacgacgtgaccgacgagctgccactgcccccgggctgggagatgaccttcacggccactggccagaggtacttcctcaatcacatagaaaaaatcaccacatggcaagaccctaggaaggcgatgaatcagcctctgaatcatatgaacctccaccctgccgtcagttccacaccagtgcctcagaggtccatggcagtatcccagccaaatctcgtgatgaatcaccaacaccagcagcagatggcccccagtaccctgagccagcagaaccaccccactcagaacccacccgcagggctcatgagtatgcccaatgcgctgaccactcagcagcagcagcagcagaaactgcggcttcagagaatccagatggagagagaaaggattcgaatgcgccaagaggagctcatgaggcaggaagctgccctctgtcgacagctccccatggaagctgagactcttgccccagttcaggctgctgtcaacccacccacgatgaccccagacatgagatccatcactaataatagctcagatcctttcctcaatggagggccatatcattcgagggagcagagcactgacagtggcctggggttagggtgctacagtgtccccacaactccggaggacttcctcagcaatgtggatgagatggatacaggagaaaacgcaggacaaacacccatgaacatcaatccccaacagacccgtttccctgatttccttgactgtcttccaggaacaaacgttgacttaggaactttggaatctgaagacctgatccccctcttcaatgatgtagagtctgctctgaacaaaagtgagccctttctaacctggctg

SEQ ID NO: 4 - DNA, 1203 bp, Homo sapiens
  ref <308>: NCBI/ 25937
  ref <309>: 2018-04-16
  ref <313>: (1)..(1203)
atgaatccggcctcggcgccccctccgctcccgccgcctgggcagcaagtgatccacgtcacgcaggacctagacacagacctcgaagccctcttcaactctgtcatgaatccgaagcctagctcgtggcggaagaagatcctgccggagtctttctttaaggagcctgattcgggctcgcactcgcgccagtccagcaccgactcgtcgggcggccacccggggcctcgactggctgggggtgcccagcatgtccgctcgcactcgtcgcccgcgtccctgcagctgggcaccggcgcgggtgctgcgggtagccccgcgcagcagcacgcgcacctccgccagcagtcctacgacgtgaccgacgagctgccactgcccccgggctgggagatgaccttcacggccactggccagaggtacttcctcaatcacatagaaaaaatcaccacatggcaagaccctaggaaggcgatgaatcagcctctgaatcatatgaacctccaccctgccgtcagttccacaccagtgcctcagaggtccatggcagtatcccagccaaatctcgtgatgaatcaccaacaccagcagcagatggcccccagtaccctgagccagcagaaccaccccactcagaacccacccgcagggctcatgagtatgcccaatgcgctgaccactcagcagcagcagcagcagaaactgcggcttcagagaatccagatggagagagaaaggattcgaatgcgccaagaggagctcatgaggcaggaagctgccctctgtcgacagctccccatggaagctgagactcttgccccagttcaggctgctgtcaacccacccacgatgaccccagacatgagatccatcactaataatagctcagatcctttcctcaatggagggccatatcattcgagggagcagagcactgacagtggcctggggttagggtgctacagtgtccccacaactccggaggacttcctcagcaatgtggatgagatggatacaggagaaaacgcaggacaaacacccatgaacatcaatccccaacagacccgtttccctgatttccttgactgtcttccaggaacaaacgttgacttaggaactttggaatctgaagacctgatccccctcttcaatgatgtagagtctgctctgaacaaaagtgagccctttctaacctggctgtaa

SEQ ID NO: 5 - protein, 488 aa, Homo sapiens
MDPGQQPPPQPAPQGQGQPPSQPPQGQGPPSGPGQPAPAATQAAPQAPPAGHQIVHVRGDSETDLEALFNAVMNPKTANVPQTVPMRLRKLPDSFFKPPEPKSHSRQASTDAGTAGALTPQHVRAHASPASLQLGAVSPGTLTPTGVVSGPAATPTAQHLRQSSFEIPDDVPLPAGWEMAKTSSGQRYFLNHIDQTTTWQDPRKAMLSQMNVTAPTSPPVQQNMMNSASGPLPDGWEQAMTQDGEIYYINHKNKTTSWLDPRLDPRFAMNQRISQSAPVKQPPPLAPQSPQGGVMGGSNSNQQQQMRLQQLQMEKERLRLKQQELLRQELALRSQLPTLEQDGGTQNPVSSPGMSQELRTMTTNSSDPFLNSGTYHSRDESTDSGLSMSSYSVPRTPDDFLNSVDEMDTGDTINQSTLPSQQNRFPDYLEAIPGTNVDLGTLEGDGMNIEGEELMPSLQEALSSDILNDMESVLAATKLDKESFLTWL

SEQ ID NO: 6 - protein, 488 aa, Homo sapiens
  ref <308>: NCBI/ NP_001181973.1
  ref <309>: 2018-03-29
  ref <313>: (1)..(488)
MDPGQQPPPQPAPQGQGQPPSQPPQGQGPPSGPGQPAPAATQAAPQAPPAGHQIVHVRGDSETDLEALFNAVMNPKTANVPQTVPMRLRKLPDSFFKPPEPKSHSRQASTDAGTAGALTPQHVRAHSSPASLQLGAVSPGTLTPTGVVSGPAATPTAQHLRQSSFEIPDDVPLPAGWEMAKTSSGQRYFLNHIDQTTTWQDPRKAMLSQMNVTAPTSPPVQQNMMNSASGPLPDGWEQAMTQDGEIYYINHKNKTTSWLDPRLDPRFAMNQRISQSAPVKQPPPLAPQSPQGGVMGGSNSNQQQQMRLQQLQMEKERLRLKQQELLRQELALRSQLPTLEQDGGTQNPVSSPGMSQELRTMTTNSSDPFLNSGTYHSRDESTDSGLSMSSYSVPRTPDDFLNSVDEMDTGDTINQSTLPSQQNRFPDYLEAIPGTNVDLGTLEGDGMNIEGEELMPSLQEALSSDILNDMESVLAATKLDKESFLTWL

SEQ ID NO: 7 - protein, 472 aa, Mus musculus
  ref <308>: NCBI/NP_001164618.1
  ref <309>: 2018-04-08
  ref <313>: (1)..(472)
MEPAQQPPPQPAPQGPAPPSVSPAGTPAAPPAPPAGHQVVHVRGDSETDLEALFNAVMNPKTANVPQTVPMRLRKLPDSFFKPPEPKSHSRQASTDAGTAGALTPQHVRAHSSPASLQLGAVSPGTLTASGVVSGPAAAPAAQHLRQSSFEIPDDVPLPAGWEMAKTSSGQRYFLNHNDQTTTWQDPRKAMLSQLNVPAPASPAVPQTLMNSASGPLPDGWEQAMTQDGEVYYINHKNKTTSWLDPRLDPRFAMNQRITQSAPVKQPPPLAPQSPQGGVLGGGSSNQQQQIQLQQLQMEKERLRLKQQELFRQELALRSQLPTLEQDGGTPNAVSSPGMSQELRTMTTNSSDPFLNSGTYHSRDESTDSGLSMSSYSIPRTPDDFLNSVDEMDTGDTISQSTLPSQQSRFPDYLEALPGTNVDLGTLEGDAMNIEGEELMPSLQEALSSEILDVESVLAATKLDKESFLTWL

SEQ ID NO: 8 - protein, 448 aa, Gallus gallus
  ref <308>: NCBI/NP_990574.1
  ref <309>: 2017-11-01
  ref <313>: (1)..(448)
MDPGQPQPQQPPQAAQPPAPQQAAPQPPGAGSGAPGGAAQPPGAGPPPAGHQIVHVRGDSETDLEALFNAVMNPKGANVPHTLPMRLRKLPDSFFKPPEPKAHSRQASTDAGTAGALTPQHVRAHSSPASLQLGAVSPGTLTPSGVVTGPGAPSSQHLRQSSFEIPDDVPLPPGWEMAKTPSGQRYFLNHIDQTTTWQDPRKAMLSQMNVTAPTSPPVQQNLMNSASAMNQRISQSAPVKQPPPLAPQSPQGGVMGGSSSNQQQQMRLQQLQMEKERLRLKHQELLRQELALRSQLPTMEQDGGSQNPVSSPGMSQELRTMTTNSSDPFLNSGTYHSRDESTDSGLSMSSYSVPRTPDDFLNSVDEMDTGDSISQSNIPSHQNRFPDYLEAIPGTNVDLGTLEGDGMNIEGEELMPSLQEALSSDILNDMESVLAATKPDKESFLTWL

SEQ ID NO: 9 - protein, 505 aa, Sus scrofa
  misc_feature (48)..(48): Xaa can be any naturally occurring amino acid
  ref <308>: NCBI/XP_020918365.1
  ref <309>: 2017-05-13
  ref <313>: (1)..(505)
MDPGQQQPPPQPAPQGQGQPPAQPPQGQGPPSGPGQPAPPGSQAATQXPPAGHQIVHVRGDSETDLEALFNAVMNPKTANVPQTVPMRLRKLPDSFFKPPEPKSHSRQASTDAGTAGALTPQHVRAHSSPASLQLGAISPGTLTPTGVVSGPAATPTAQHLRQSSFEIPDDVPLPAGWEMAKTSSGQRYFLNHIDQTTTWQDPRKAMLSQMNVTAPTSPPVQQNMMNSASGPLPDGWEQAMTQDGEIYYINHKNKTTSWLDPRLDPRFAMNQRISQSAPVKQPPPLAPQSPQGGVMGGGSSNQQQQMRLQQLQMEKERLRLKQQELLRQAMRNINPSTANSPKCQELALRSQLPTLEQDGGTQNPVSSPGMSQELRTMTTNSSDPFLNSGTYHSRDESTDSGLSMSSYSVPRTPDDFLNSVDEMDTGDTINQSTLPSQQNRFPDYLEAIPGTNVDLGTLEGDGMNIEGEELMPSLQEALSSDILNDMESVLAATKLDKESFLTWL

SEQ ID NO: 10 - protein, 432 aa, Bos taurus
  ref <308>: NCBI/XP_015321922.1
  ref <309>: 2016-01-26
  ref <313>: (1)..(432)
MNPKTANVPQTVPMRLRKLPDSFFKPPEPKSHSRQASTDAGTAGALTPQHVRAHSSPASLQLGAVSPGTLTPTGVVSGPAAAPAAQHLRQSSFEIPDDVPLPAGWEMAKTSSGQRYFLNHIDQTTTWQDPRKAMLSQMNVTAPTSPPVQQNMMNSASGPLPDGWEQAMTQDGEIYYINHKNKTTSWLDPRLDPRFAMNQRISQSAPVKQPPPLAPQSPQGGVLGGGSSNQQQQMRLQQLQMEKERLRLKQQELLRQAMRNINPSTANSPKCQELALRSQLPTLEQDGGTQNPVSSPGMSQELRTMTTNSSDPFLNSGTYHSRDESTDSGLSMSSYSVPRTPDDFLNSVDEMDTGDTINQSTLPSQQNRFPDYLEAIPGTNVDLGTLEGDGMNIEGEELMPSLQEALSSDILNDMESVLAATKLDKESFLTWL

SEQ ID NO: 11 - protein, 437 aa, Oreochromis niloticus
  ref <308>: NCBI/XP_003450207.1
  ref <309>: 2016-12-05
  ref <313>: (1)..(437)
MDPSQHNPPAGHQIVHVRGDSETDLEALFNAVMNPKVNTVPHSVPMRMRKLPDSFFKPPEPKSHSRQASTDAGSGGVLIPHHVRAHSSPASLQLGAVSGGSLSGMGSTGASPQHLRQSSYEIPDDMPLPDGWEMAKTASGQRYFLNHIDQTTTWQDPRKAMLQMNQPPPPSSVPVQPQPIMNPASGPLPDGWEQAITAEGEIYYINHKNKTTSWLDPRLEPRYALNQQRISQSAPVKPPGQLPPSISGVMGSNNQMRLQQIEKERLRLKQQELLRQRPQELALRNQLPTSMDQDGSTNPVSSPMAQDARTMTANSSDPFLNSGTYHSRDESTDSGLSMSSYSVPRTPDDFLNSVDEMDTGDPLAPSMATQPSRFPDYLDTIPGTDVDLGTLEGESMAVEGEELMPSLQEALSSDILNDMESVLAATKLDKESFLTWL

SEQ ID NO: 12 - protein, 400 aa, Homo sapiens
MNPASAPPPLPPPGQQVIHVTQDLDTDLEALFNSVMNPKPSSWRKKILPESFFKEPDSGSHSRQSSTDSSGGHPGPRLAGGAQHVRSHASPASLQLGTGAGAAGSPAQQHAHLRQQSYDVTDELPLPPGWEMTFTATGQRYFLNHIEKITTWQDPRKAMNQPLNHMNLHPAVSSTPVPQRSMAVSQPNLVMNHQHQQQMAPSTLSQQNHPTQNPPAGLMSMPNALTTQQQQQQKLRLQRIQMERERIRMRQEELMRQEAALCRQLPMEAETLAPVQAAVNPPTMTPDMRSITNNSSDPFLNGGPYHSREQSTDSGLGLGCYSVPTTPEDFLSNVDEMDTGENAGQTPMNINPQQTRFPDFLDCLPGTNVDLGTLESEDLIPLFNDVESALNKSEPFLTWL

SEQ ID NO: 13 - protein, 400 aa, Homo sapiens
  ref <308>: NCBI/25937
  ref <309>: 2018-04-16
  ref <313>: (1)..(400)
MNPASAPPPLPPPGQQVIHVTQDLDTDLEALFNSVMNPKPSSWRKKILPESFFKEPDSGSHSRQSSTDSSGGHPGPRLAGGAQHVRSHSSPASLQLGTGAGAAGSPAQQHAHLRQQSYDVTDELPLPPGWEMTFTATGQRYFLNHIEKITTWQDPRKAMNQPLNHMNLHPAVSSTPVPQRSMAVSQPNLVMNHQHQQQMAPSTLSQQNHPTQNPPAGLMSMPNALTTQQQQQQKLRLQRIQMERERIRMRQEELMRQEAALCRQLPMEAETLAPVQAAVNPPTMTPDMRSITNNSSDPFLNGGPYHSREQSTDSGLGLGCYSVPTTPEDFLSNVDEMDTGENAGQTPMNINPQQTRFPDFLDCLPGTNVDLGTLESEDLIPLFNDVESALNKSEPFLTWL

SEQ ID NO: 14 - protein, 395 aa, Mus musculus
  ref <308>: NCBI/NP_033560.1
  ref <309>: 2016-04-26
  ref <313>: (1)..(395)
MNPSSVPHPLPPPGQQVIHVTQDLDTDLEALFNSVMNPKPSSWRKKILPESFFKEPDSGSHSRQSSTDSSGGHPGPRLAGGAQHVRSHSSPASLQLGTGAGAAGGPAQQHAHLRQQSYDVTDELPLPPGWEMTFTATGQRYFLNHIEKITTWQDPRKVMNQPLNHVNLHPSITSTSVPQRSMAVSQPNLAMNHQHQQVVATSLSPQNHPTQNQPTGLMSVPNALTTQQQQQQKLRLQRIQMERERIRMRQEELMRQEAALCRQLPMETETMAPVNTPAMSTDMRSVTNSSSDPFLNGGPYHSREQSTDSGLGLGCYSVPTTPEDFLSNMDEMDTGENSGQTPMTVNPQQTRFPDFLDCLPGTNVDLGTLESEDLIPLFNDVESALNKSEPFLTWL

SEQ ID NO: 15 - protein, 386 aa, Gallus gallus
  ref <308>: NCBI/XP_003641834.1
  ref <309>: 2018-01-04
  ref <313>: (1)..(386)
MNPSPAAPPPGQQVIHITQDLDTELEALFNAVMNPRPSSWRKKILPESFFKEPDSGSHSRQSSTDSGGPPPRPVAAQHVRSHSSPASLVGSAAAPQHGHLRQRSYDVTDELPLPPGWEMALTHTGQRYFLNHIEKITTWQDPRKTMNQPLNHMSHHPAATSTPVPQRSMAMSQPNLVMNHQHQITGNTSISQQSCPSQTPQPGLLNMPSALTAQQQQQQKLRLQRIQMERERIRMRQEELLRQEAALCRQLPMDSENMTAVQTAVSTAAMTQDMRSITNNGSDPFLNSGPYHSREQSTDSGLGLGCYSIPTTPEDFLSNVDEMDTGETVAQTTVNINAQQTRFPDFLDCLPGTNVDLGTLESEDLIPILNDVESVLSKNEPFLTWL

SEQ ID NO: 16 - protein, 399 aa, Sus scrofa
  misc_feature (129)..(129): Xaa can be any naturally occurring amino acid
  ref <308>: NCBI/XP_013847805.2
  ref <309>: 2017-05-13
  ref <313>: (1)..(399)
MNPASAPPPLPPPGQQVIHVTQDLDTDLEALFNSVMNPKPSSWRKKILPESFFKEPDSGSHSRQSSTDSSGGHPGPRLAGGAQHVRSHSSPASLQLGTGAGAAGNPAQQHAHLRQQSYDVTDELPLPPXWEMTFTATGQRYFLNHIEKITTWQDPRKAMNQPLNHMNLHPAATSTPAPQRSMAVSQPNLVMNHHQQQMAPSSLSQQSHPPQNPPAGLMNMPNALTTQQQQQQKLRLQRIQMERERIRMRQEELMRQEAALCRQLPMEAETLPTVQAAVNPPAMTPDMRSITNNSSDPFLNGGPYHSREQSTDSGLGLGCYSVPTTPEDFLSNVDEMDTGENAGPTPMNINPQQTRFPDFLDCLPGTNVDLGTLESEDLIPLFNDVESALNKSEPFLTWL

SEQ ID NO: 17 - protein, 400 aa, Bos taurus
  ref <308>: NCBI/NP_001179976.1
  ref <309>: 2015-01-04
  ref <313>: (1)..(400)
MNPASAPPPLPPPGQQVIHVTQDLDTDLEALFNSVMNPKPSSWRKKILPESFFKEPDSGSHSRQSSTDSSGGHPGPRLAGGAQHVRSHSSPASLQLGTGAGAAVSPAQQHAHLRQQSYDVTDELPLPPGWEMTFTATGQRYFLNHIEKITTWQDPRKAMNQPLNHMNLHPAATSTPAPQRSMAVSQPNLVMNHQHQQQMAPSSLSQQNHPPQNPSAGLMSMPNALTTQQQQQQKLRLQRIQMERERIRMRQEELMRQEAALCRQLPMEAETLATVQAAVNPPAMTPDMRSITNNSSDPFLNGGPYHSREQSTDSGLGLGCYSVPTTPEDFLSNVDEMDTGENTGQTPMNINPQQTRFPDFLDCLPGTNVDLGTLESEDLIPLFNDVESALNKSEPFLTWL

SEQ ID NO: 18 - protein, 391 aa, Danio rerio
  ref <308>: NCBI/NP_001032785.1
  ref <309>: 2017-08-06
  ref <313>: (1)..(391)
MSGNPLQPIPGHQVIHVAKDLDTDLEALFNSVMNPKPSSWRNKDMPQSFFQEPDSGSHSRQSSADSGSLPPRVHFRSRSSPASLQLPAGSVSGPSPGRLHSHTRHQSCDVAEELPLPPGWEMAFTPNGQKYFLNHIEKITTWHDPRKSMTPSVAQLSLHNQVSNTASIQQRSMALSQPNLVLNQQAHQQQQQHLQQQQQQVPVQVPVQAPQQQSSQPMMNLSAQQHQQKMRLQRIQMERERIQRRQEELMRQEVALRQLPMDSDNLPPVAPAIGSPAMSAGNMPNNSADPFLNSGPYHSREQSTDSGLGLGCYSIPTTPEDFLNNMEDMDTGENMVPVSMNVPPQSRFPDFLDSMPGTNVDLGTLEGTDLMPILNDVESVLNKSEPFLTWL

SEQ ID NO: 19 - protein, 395 aa, Drosophila melanogaster
  ref <308>: NCBI/NP_726414.3
  ref <309>: 2017-08-06
  ref <313>: (1)..(395)
MLTTMSASSNTNSLIEKEIDDEDMLSPIKSNNLVVRVNQDTDDNLQALFDSVLNPGDAKRPLQLPLRMRKLPNSFFTPPAPSHSRANSADSTYDAGSQSSINIGNKASIVQQPDGQSPIAAIPQLQIQPSPQHSRLAIHHSRARSSPASLQQNYNVRARSDAAAANNPNANPSSQQQPAGPTFPENSAQEFPSGAPASSAIDLDAMNTCMSQDIPMSMQTVHKKQRSYDVISPIQLNRQLGALPPGWEQAKTNDGQIYYLNHTTKSTQWEDPRIQYRQQQQILMAERIKQNDVLQTTKQTTTSTIANNLGPLPDGWEQAVTESGDLYFINHIDRTTSWNDPRMQSGLSVLDCPDNLVSSLQIEDNLCSNLFNDAQAIVNPPSSHKPDDLEWYKIN

SEQ ID NO: 20 - DNA, 19 bp, Homo sapiens
cagcagcaacagatgcgac

SEQ ID NO: 21 - DNA, 25 bp, Homo sapiens
cagccaaaacagactccatgtcatt

SEQ ID NO: 22 - DNA, 20 bp, Homo sapiens
agctcagcatcttcgacagt

SEQ ID NO: 23 - DNA, 22 bp, Homo sapiens
tcaggaagtcatctggggttcg

SEQ ID NO: 24 - DNA, 31 bp, Artificial Sequence
  Synthetically constructed primer
  misc_feature (7)..(7): n is a, c, g, or t
  misc_feature (10)..(10): n is a, c, g, or t
thacatnrrncccatgcgcattaaggtggtc

SEQ ID NO: 25 - DNA, 20 bp, Artificial Sequence
  Synthetically constructed primer
tcgaccggtacgtagtcaca

SEQ ID NO: 26 - DNA, 20 bp, Artificial Sequence
  Synthetically constructed primer
acctacgaagatggaggcgt

SEQ ID NO: 27 - DNA, 19 bp, Artificial Sequence
  Synthetically constructed primer
gcgtgttccctctgaacga

SEQ ID NO: 28 - DNA, 22 bp, Artificial Sequence
  Synthetically constructed primer
tccgcgttacataacttacggt

SEQ ID NO: 29 - DNA, 20 bp, Artificial Sequence
  Synthetically constructed primer
cccgtgagtcaaaccgctat

SEQ ID NO: 30 - DNA, 20 bp, Artificial Sequence
  Synthetically constructed primer
aagtacgccccctattgacg

SEQ ID NO: 31 - DNA, 20 bp, Artificial Sequence
  Synthetically constructed primer
tacacgcctaccgcccattt